European Patent Application EP 4 582 093 A1, published July 9, 2025. Title: A FERTILITY-ENHANCING COMPOSITION OF RUMINANTS. Applicant: Hokkaido University. Application JP. The sequence listing filed with the application follows.

SEQUENCE LISTING (8 sequences)

SEQ ID NO: 1 - protein, 7 aa, Bos taurus
SVAYGLK

SEQ ID NO: 2 - protein, 11 aa, Bos taurus
GRGDSVAYGLK

SEQ ID NO: 3 - protein, 5 aa, Bos taurus
GRGDS

SEQ ID NO: 4 - protein, 278 aa, Bos taurus
MRIAVICFCLLGIASALPVKPTSSGSSEEKQLNNKYPDAVATWLKPDPSQKQTFLAPQNSVSSEETDDNKQNTLPSKSNESPEQTDDLDDDDDNSQDVNSNDSDDAETTDDPDHSDESHHSDESDEVDFPTDIPTIAVFTPFIPTESANDGRGDSVAYGLKSRSKKFRRSNVQSPDATEEDFTSHIESEEMHDAPKKTSQLTDHSKETNSSELSKELTPKAKDKNKHSNLIESQENSKLSQEFHSLEDKLDLDHKSEEDKHLKIRISHELDSASSEVN

SEQ ID NO: 5 - DNA, 39 bp, synthetic construct
  source 1..39: mol_type = other DNA
gccgcgcggcagccatatgctgccggttaaaccgaccag

SEQ ID NO: 6 - DNA, 39 bp, synthetic construct
  source 1..39: mol_type = other DNA
cgagtgcggccgcaagcttttaattcacttcactgcttg

SEQ ID NO: 7 - protein, 21 aa, synthetic construct
MGSSHHHHHHSSGLVPRGSHM

SEQ ID NO: 8 - protein, 11 aa, synthetic construct
GRGESVAYGLK